European Patent Specification EP 3 976 809 B1, published June 5, 2024. Title: VARIANTS OF TERMINAL DEOXYNUCLEOTIDYL TRANSFERASE AND USES THEREOF. Applicant: DNA Script SAS. The sequence listing filed with the application follows.

SEQUENCE LISTING (35 sequences)

SEQ ID NO: 1 - protein, 510 aa, Mus musculus
MDPLQAVHLGPRKKRPRQLGTPVASTPYDIRFRDLVLFILEKKMGTTRRAFLMELARRKGFRVENELSDSVTHIVAENNSGSDVLEWLQLQNIKASSELELLDISWLIECMGAGKPVEMMGRHQLVVNRNSSPSPVPGSQNVPAPAVKKISQYACQRRTTLNNYNQLFTDALDILAENDELRENEGSCLAFMRASSVLKSLPFPITSMKDTEGIPCLGDKVKSIIEGIIEDGESSEAKAVLNDERYKSFKLFTSVFGVGLKTAEKWFRMGFRTLSKIQSDKSLRFTQMQKAGFLYYEDLVSCVNRPEAEAVSMLVKEAVVTFLPDALVTMTGGFRRGKMTGHDVDFLITSPEATEDEEQQLLHKVTDFWKQQGLLLYCDILESTFEKFKQPSRKVDALDHFQKCFLILKLDHGRVHSEKSGQQEGKGWKAIRVDLVMCPYDRRAFALLGWTGSRQFERDLRRYATHERKMMLDNHALYDRTKRVFLEAESEEEIFAHLGLDYIEPWERNA

SEQ ID NO: 2 - protein, 381 aa, Mus musculus
NSSPSPVPGSQNVPAPAVKKISQYACQRRTTLNNYNQLFTDALDILAENDELRENEGSCLAFMRASSVLKSLPFPITSMKDTEGIPCLGDKVKSIIEGIIEDGESSEAKAVLNDERYKSFKLFTSVFGVGLKTAEKWFRMGFRTLSKIQSDKSLRFTQMQKAGFLYYEDLVSCVNRPEAEAVSMLVKEAVVTFLPDALVTMTGGFRRGKMTGHDVDFLITSPEATEDEEQQLLHKVTDFWKQQGLLLYCDILESTFEKFKQPSRKVDALDHFQKCFLILKLDHGRVHSEKSGQQEGKGWKAIRVDLVMCPYDRRAFALLGWTGSRQFERDLRRYATHERKMMLDNHALYDRTKRVFLEAESEEEIFAHLGLDYIEPWERNA

SEQ ID NO: 3 - protein, 494 aa, Homo sapiens
MLPKRRRARVGSPSGDAASSTPPSTRFPGVAIYLVEPRMGRSRRAFLTGLARSKGFRVLDACSSEATHVVMEETSAEEAVSWQERRMAAAPPGCTPPALLDISWLTESLGAGQPVPVECRHRLEVAGPRKGPLSPAWMPAYACQRPTPLTHHNTGLSEALEILAEAAGFEGSEGRLLTFCRAASVLKALPSPVTTLSQLQGLPHFGEHSSRVVQELLEHGVCEEVERVRRSERYQTMKLFTQIFGVGVKTADRWYREGLRTLDDLREQPQKLTQQQKAGLQHHQDLSTPVLRSDVDALQQVVEEAVGQALPGATVTLTGGFRRGKLQGHDVDFLITHPKEGQEAGLLPRVMCRLQDQGLILYHQHQHSCCESPTRLAQQSHMDAFERSFCIFRLPQPPGAAVGGSTRPCPSWKAVRVDLVVAPVSQFPFALLGWTGSKLFQRELRRFSRKEKGLWLNSHGLFDPEQKTFFQAASEEDIFRHLGLEYLPPEQRNA

SEQ ID NO: 4 - protein, 401 aa, Homo sapiens
TMGSSHHHHHHSSGLVPRGSHMSPSPVPGSQNVPAPAVKKISQYACQRRTTLNNYNQLFTDALDILAENDELRENEGSCLAFMRASSVLKSLPFPITSMKDTEGIPCLGDKVKSIIEGIIEDGESSEAKAVLNDERYKSFKLFTSVFGVGLKTAEKWFRMGFRTLSKIQSDKSLRFTQMQKAGFLYYEDLVSCVNRPEAEAVSMLVKEAVVTFLPDALVTMTGGFRRGKMTGHDVDFLITSPEATEDEEQQLLHKVTDFWKQQGLLLYCDILESTFEKFKQPSRKVDALDHFQKCFLILKLDHGRVHSEKSGQQEGKGWKAIRVDLVMCPYDRRAFALLGWTGSRQFERDLRRYATHERKMMLDNHALYDRTKRVFLEAESEEEIFAHLGLDYIEPWERNA

SEQ ID NO: 5 - DNA, 20 bp, Artificial Sequence
  t7-pro primer
taatacgactcactataggg

SEQ ID NO: 6 - DNA, 19 bp, Artificial Sequence
  T7-ter primer
gctagttattgctcagcgg

SEQ ID NO: 7 - DNA, 18 bp, Artificial Sequence
  primer
aaaaaaaaaaaaaagggg

SEQ ID NO: 8 - DNA, 20 bp, Artificial Sequence
  primer
ttttttttttttaaataagg

SEQ ID NO: 9 - protein, 401 aa, Artificial Sequence
  Reference TdT variant
TMGSSHHHHHHSSGLVPRGSHMSPSPVPGSQNVPAPAVKKISQYACQRRTTLNNYNQLFTDALDILAENDELRENEGSCLAFMRASSVLKSLPFPITSMKDTEGIPCLGDKVKSIIEGIIEDGESSEAKAVLNDERYKSFKLFTSVFGVGLKTAEKWFRMGFRTLSKIQSDKSLRFTQMQKAGFLYYEDLVSCVNRPEAEAVSMLVKEAVVTFLPDALVTMTGGFRRGKMTGHDVDFLITSPEATEDEEQQLLHKVTDFWKQQGLLLYCDILESTFEKFKQPSRKVDALDHFQKCFLILKLDHGRVHSEKSGQQEGKGWKAIRVDLVMCPYDRRAFALLGWTGSAQFSRDLRRYATHERKMMLDNHALYDRTKRVFLEAESEEEIFAHLGLDYIEPWERNA

SEQ ID NO: 10 - protein, 519 aa, Bos taurus
MAQQRQHQRLPMDPLCTASSGPRKKRPRQVGASMASPPHDIKFQNLVLFILEKKMGTTRRNFLMELARRKGFRVENELSDSVTHIVAENNSGSEVLEWLQVQNIRASSQLELLDVSWLIESMGAGKPVEITGKHQLVVRTDYSATPNPGFQKTPPLAVKKISQYACQRKTTLNNYNHIFTDAFEILAENSEFKENEVSYVTFMRAASVLKSLPFTIISMKDTEGIPCLGDKVKCIIEEIIEDGESSEVKAVLNDERYQSFKLFTSVFGVGLKTSEKWFRMGFRSLSKIMSDKTLKFTKMQKAGFLYYEDLVSCVTRAEAEAVGVLVKEAVWAFLPDAFVTMTGGFRRGKKIGHDVDFLITSPGSAEDEEQLLPKVINLWEKKGLLLYYDLVESTFEKFKLPSRQVDTLDHFQKCFLILKLHHQRVDSSKSNQQEGKTWKAIRVDLVMCPYENRAFALLGWTGSRQFERDIRRYATHERKMMLDNHALYDKTKRVFLKAESEEEIFAHLGLDYIEPWERN

SEQ ID NO: 11 - protein, 380 aa, Bos taurus
DYSATPNPGFQKTPPLAVKKISQYACQRKTTLNNYNHIFTDAFEILAENSEFKENEVSYVTFMRAASVLKSLPFTIISMKDTEGIPCLGDKVKCIIEEIIEDGESSEVKAVLNDERYQSFKLFTSVFGVGLKTSEKWFRMGFRSLSKIMSDKTLKFTKMQKAGFLYYEDLVSCVTRAEAEAVGVLVKEAVWAFLPDAFVTMTGGFRRGKKIGHDVDFLITSPGSAEDEEQLLPKVINLWEKKGLLLYYDLVESTFEKFKLPSRQVDTLDHFQKCFLILKLHHQRVDSSKSNQQEGKTWKAIRVDLVMCPYENRAFALLGWTGSRQFERDIRRYATHERKMMLDNHALYDKTKRVFLKAESEEEIFAHLGLDYIEPWERNA

SEQ ID NO: 12 - protein, 509 aa, Homo sapiens
MDPPRASHLSPRKKRPRQTGALMASSPQDIKFQDLVVFILEKKMGTTRRAFLMELARRKGFRVENELSDSVTHIVAENNSGSDVLEWLQAQKVQVSSQPELLDVSWLIECIRAGKPVEMTGKHQLVVRRDYSDSTNPGPPKTPPIAVQKISQYACQRRTTLNNCNQIFTDAFDILAENCEFRENEDSCVTFMRAASVLKSLPFTIISMKDTEGIPCLGSKVKGIIEEIIEDGESSEVKAVLNDERYQSFKLFTSVFGVGLKTSEKWFRMGFRTLSKVRSDKSLKFTRMQKAGFLYYEDLVSCVTRAEAEAVSVLVKEAVWAFLPDAFVTMTGGFRRGKKMGHDVDFLITSPGSTEDEEQLLQKVMNLWEKKGLLLYYDLVESTFEKLRLPSRKVDALDHFQKCFLIFKLPRQRVDSDQSSWQEGKTWKAIRVDLVLCPYERRAFALLGWTGSRQFERDLRRYATHERKMILDNHALYDKTKRIFLKAESEEEIFAHLGLDYIEPWERNA

SEQ ID NO: 13 - protein, 380 aa, Homo sapiens
DYSDSTNPGPPKTPPIAVQKISQYACQRRTTLNNCNQIFTDAFDILAENCEFRENEDSCVTFMRAASVLKSLPFTIISMKDTEGIPCLGSKVKGIIEEIIEDGESSEVKAVLNDERYQSFKLFTSVFGVGLKTSEKWFRMGFRTLSKVRSDKSLKFTRMQKAGFLYYEDLVSCVTRAEAEAVSVLVKEAVWAFLPDAFVTMTGGFRRGKKMGHDVDFLITSPGSTEDEEQLLQKVMNLWEKKGLLLYYDLVESTFEKLRLPSRKVDALDHFQKCFLIFKLPRQRVDSDQSSWQEGKTWKAIRVDLVLCPYERRAFALLGWTGSRQFERDLRRYATHERKMILDNHALYDKTKRIFLKAESEEEIFAHLGLDYIEPWERNA

SEQ ID NO: 14 - protein, 506 aa, Gallus gallus
MERIRPPTVVSQRKRQKGMYSPKLSCGYEIKFNKLVIFIMQRKMGMTRRTFLMELARSKGFRVESELSDSVTHIVAENNSYPEVLDWLKGQAVGDSSRFEILDISWLTACMEMGRPVDLEKKYHLVEQAGQYPTLKTPESEVSSFTASKVSQYSCQRKTTLNNCNKKFTDAFEIMAENYEFKENEIFCLEFLRAASVLKSLPFPVTRMKDIQGLPCMGDRVRDVIEEIIEEGESSRAKDVLNDERYKSFKEFTSVFGVGVKTSEKWFRMGLRTVEEVKADKTLKLSKMQRAGFLYYEDLVSCVSKAEADAVSSIVKNTVCTFLPDALVTITGGFRRGKKIGHDIDFLITSPGQREDDELLHKGLLLYCDIIESTFVKEQIPSRHVDAMDHFQKCFAILKLYQPRVDNSSYNMSKKCDMAEVKDWKAIRVDLVITPFEQYAYALLGWTGSRQFGRDLRRYATHERKMMLDNHALYDKRKRVFLKAGSEEEIFAHLGLDYVEPWERNA

SEQ ID NO: 15 - protein, 376 aa, Gallus gallus
QYPTLKTPESEVSSFTASKVSQYSCQRKTTLNNCNKKFTDAFEIMAENYEFKENEIFCLEFLRAASVLKSLPFPVTRMKDIQGLPCMGDRVRDVIEEIIEEGESSRAKDVLNDERYKSFKEFTSVFGVGVKTSEKWFRMGLRTVEEVKADKTLKLSKMQRAGFLYYEDLVSCVSKAEADAVSSIVKNTVCTFLPDALVTITGGFRRGKKIGHDIDFLITSPGQREDDELLHKGLLLYCDIIESTFVKEQIPSRHVDAMDHFQKCFAILKLYQPRVDNSSYNMSKKCDMAEVKDWKAIRVDLVITPFEQYAYALLGWTGSRQFGRDLRRYATHERKMMLDNHALYDKRKRVFLKAGSEEEIFAHLGLDYVEPWERNA

SEQ ID NO: 16 - protein, 518 aa, Monodelphis domestica
MHRIRTIDSDFGKKRQKKMDNHISSMIYEIKFHEFVLFILEKKMGATRRTFLTDLARKKGFRVENELSNSVTHIVAENNSGSDVLAWLKTHKMEKTTQFELLDISWLIECMKVGKPVDTKGKYQLMESRVDSANPDPTAGTLNILPPTTKTISQYACQRRTTINNHNQRFTDAFEILAKNYEFKENDDTCLTFMRAISVLKCLPFEVVSLKDTEGLPWIGDEVKGIMEEIIEDGESLEVQAVLNDERYQSFKLFTSVFGVGLKTADKWYRMGFRTLNKIRSDKTLKLTKMQKAGLCYYEDLIDCVSKAEADAVSLLVQDAVWTFLPDALVTITGGFRRGKEFGHDVDFLITSPGAEKEQEDQLLQKVTNLWKKQGLLLYCDLIESTFEDLKLPSRKIDALDHFQKCFLILKLYHHKEDKRKWEMPTGSNESEAKSWKAIRVDLVVCPYDRYAFALLGWSGSRQFERDLRRYATHEKKMMLDNHALYDKTKKIFLKAKSEEEIFAHLGLEYIQPSERNA

SEQ ID NO: 17 - protein, 387 aa, Monodelphis domestica
SANPDPTAGTLNILPPTTKTISQYACQRRTTINNHNQRFTDAFEILAKNYEFKENDDTCLTFMRAISVLKCLPFEVVSLKDTEGLPWIGDEVKGIMEEIIEDGESLEVQAVLNDERYQSFKLFTSVFGVGLKTADKWYRMGFRTLNKIRSDKTLKLTKMQKAGLCYYEDLIDCVSKAEADAVSLLVQDAVWTFLPDALVTITGGFRRGKEFGHDVDFLITSPGAEKEQEDQLLQKVTNLWKKQGLLLYCDLIESTFEDLKLPSRKIDALDHFQKCFLILKLYHHKEDKRKWEMPTGSNESEAKSWKAIRVDLVVCPYDRYAFALLGWSGSRQFERDLRRYATHEKKMMLDNHALYDKTKKIFLKAKSEEEIFAHLGLEYIQPSERNA

SEQ ID NO: 18 - protein, 512 aa, Elephantulus edwardii
MDPLQMACTGPRKKRARQMDTSMGSTQDIKFQDLVLFILEKKMGTTRRAFLMELARRKGFRVENELSDSVTHIVAENNSGSDVLEWLQVQKIKASSQLELLDVSWLIECMGAGKLVEITGKHQLVSIMVRGDCPASHDSSPQKTESAAVQKISQYACQRRTTLNNHNHIFTDAFEILAENCEFRENEGSYVTYMRAASVLKSLPFSIISMKDTEGIPCLADKVKCVIEEIIEDGESSEVKAVLNDERYKSFKLFTSVFGVGLKTAEKWFRLGFRTLSGIMNDKTLKLTHMQKAGFLYYEDLVSCVTRAEAEAVGVLVKEAVWAFLPDAIVTMTGGFRRGKKVGHDVDFLITSPEATEEQEQQLLHKVITFWEKEGLLLYCDLYESTFEKLKMPSRKVDALDHFQKCFLILKLHRECVDDGTSSQLQGKTWKAIRVDLVVCPYECRAFALLGWTGSPQFERDLRRYATHERKMMLDNHALYDKTKRKFLSADSEEDIFAHLGLDYIEPWERNA

SEQ ID NO: 19 - protein, 381 aa, Elephantulus edwardii
DCPASHDSSPQKTESAAVQKISQYACQRRTTLNNHNHIFTDAFEILAENCEFRENEGSYVTYMRAASVLKSLPFSIISMKDTEGIPCLADKVKCVIEEIIEDGESSEVKAVLNDERYKSFKLFTSVFGVGLKTAEKWFRLGFRTLSGIMNDKTLKLTHMQKAGFLYYEDLVSCVTRAEAEAVGVLVKEAVWAFLPDAIVTMTGGFRRGKKVGHDVDFLITSPEATEEQEQQLLHKVITFWEKEGLLLYCDLYESTFEKLKMPSRKVDALDHFQKCFLILKLHRECVDDGTSSQLQGKTWKAIRVDLVVCPYECRAFALLGWTGSPQFERDLRRYATHERKMMLDNHALYDKTKRKFLSADSEEDIFAHLGLDYIEPWERNA

SEQ ID NO: 20 - protein, 506 aa, Artificial Sequence
  Python bivittatus
MNKMKTSDFSPMRKRQKRMQIAAPLSSYKIEFKDIIIFIVERKMGMTRRMFLMDLARRKGFRVENELSDLVTHVVAENNSCSEILKWLQKHNVEDSSRFRILDIRWLTACMEVGRPVDSEKYQLPEDEDRSVTSDLDRDSISEYACQRRTTLKNYNQKFTDAFEILAENYEFNENKGFCTAFRRAASVLKCLPFTIVQVHDIEGVPWMGKQVKGIIEDIIEEGESSKVKAVLDNENYRSVKLFTSVFGVGLKTSDKWYRMGLRTLEEVKRDKNLKLTRMQKAGFLHYDDLTSCVSKAEADAASLIVQDVVWKIVPNAIVTIAGGFRRGKQTGHDVDFLITVPGSKQEEEELLHTVIDIWKKQELLLYYDLIESTFEDTKLPSRKVDALDHFQKCFAILKVHKEREDKGNSIRSKAFSEEEIKDWKAIRVDLVVVPFEQYAFALLGWTGSTQFERDLRRYATHEKKMMLDNHALYDKTKKIFLNAASEEEIFAHLGLDYLEPWERNA

SEQ ID NO: 21 - protein, 387 aa, Artificial Sequence
  Python bivittatus
EKYQLPEDEDRSVTSDLDRDSISEYACQRRTTLKNYNQKFTDAFEILAENYEFNENKGFCTAFRRAASVLKCLPFTIVQVHDIEGVPWMGKQVKGIIEDIIEEGESSKVKAVLDNENYRSVKLFTSVFGVGLKTSDKWYRMGLRTLEEVKRDKNLKLTRMQKAGFLHYDDLTSCVSKAEADAASLIVQDVVWKIVPNAIVTIAGGFRRGKQTGHDVDFLITVPGSKQEEEELLHTVIDIWKKQELLLYYDLIESTFEDTKLPSRKVDALDHFQKCFAILKVHKEREDKGNSIRSKAFSEEEIKDWKAIRVDLVVVPFEQYAFALLGWTGSTQFERDLRRYATHEKKMMLDNHALYDKTKKIFLNAASEEEIFAHLGLDYLEPWERNA

SEQ ID NO: 22 - protein, 490 aa, Canis lupus
MGAEAGTWRDTGGKFLLLATEPERKFRASDACCQGPSPAGQALEETGACDSITHIVAENNSGSDVLEWLQVQNIKASSQLELLDISWLIESMGAGKPVEMTGKHQLMRRDYTASPNPELQKTLPVAVKKISQYACQRRTTLNNYNNVFTDAFEVLAENYEFRENEVFSLTFMRAASVLKSLPFTIISMKDTEGIPCLGDQVKCIIEEIIEDGESSEVKAVLNDERYQSFKLFTSVFGVGLKTSEKWFRMGFRTLSKIKSDKSLKFTPMQKAGFLYYEDLVSCVTRAEAEAVGVLVKEAVGAFLPDAFVTMTGGFRRGKKMGHDVDFLITSPGSTDEDEEQLLPKVINLWERKGLLLYCDLVESTFEKLKLPSRKVDALDHFQKCFLILKLHHQRVDGGKCSQQEGKTWKAIRVDLVMCPYERRAFALLGWTGSRQFERDLRRYASHERKMILDNHALYDKTKKIFLKAESEEEIFAHLGLDYIEPWERNA

SEQ ID NO: 23 - protein, 381 aa, Canis lupus
DYTASPNPELQKTLPVAVKKISQYACQRRTTLNNYNNVFTDAFEVLAENYEFRENEVFSLTFMRAASVLKSLPFTIISMKDTEGIPCLGDQVKCIIEEIIEDGESSEVKAVLNDERYQSFKLFTSVFGVGLKTSEKWFRMGFRTLSKIKSDKSLKFTPMQKAGFLYYEDLVSCVTRAEAEAVGVLVKEAVGAFLPDAFVTMTGGFRRGKKMGHDVDFLITSPGSTDEDEEQLLPKVINLWERKGLLLYCDLVESTFEKLKLPSRKVDALDHFQKCFLILKLHHQRVDGGKCSQQEGKTWKAIRVDLVMCPYERRAFALLGWTGSRQFERDLRRYASHERKMILDNHALYDKTKKIFLKAESEEEIFAHLGLDYIEPWERNA

SEQ ID NO: 24 - protein, 512 aa, Artificial Sequence; identical to SEQ ID NO: 18
  Condylura cristata

SEQ ID NO: 25 - protein, 382 aa, Artificial Sequence
  Condylura cristata
GDCPASHDSSPQKTESAAVQKISQYACQRRTTLNNHNHIFTDAFEILAENCEFRENEGSYVTYMRAASVLKSLPFSIISMKDTEGIPCLADKVKCVIEEIIEDGESSEVKAVLNDERYKSFKLFTSVFGVGLKTAEKWFRLGFRTLSGIMNDKTLKLTHMQKAGFLYYEDLVSCVTRAEAEAVGVLVKEAVWAFLPDAIVTMTGGFRRGKKVGHDVDFLITSPEATEEQEQQLLHKVITFWEKEGLLLYCDLYESTFEKLKMPSRKVDALDHFQKCFLILKLHRECVDDGTSSQLQGKTWKAIRVDLVVCPYECRAFALLGWTGSPQFERDLRRYATHERKMMLDNHALYDKTKRKFLSADSEEDIFAHLGLDYIEPWERNA

SEQ ID NO: 26 - protein, 508 aa, Ochotona princeps
MDSLQTGHLGPRKKRSRQTDAARTSIPQEVKFQDLVLFILEKKMGSTRRAFLMELARSKGFRVENELSDSVTHIVAENNSGSDVLEWLQVQKLKDSSQLELLDVSWLIECMRAGKPVATTGKHQLVMREEYSANPSPGPQATPAVYKISQYACQRRTTLNNHNHIFTDAFEILAENYEFKENEGCYVTYMRAASVLKSLPFTIVSMKDTEGIPCLEDKVKSIMEEIIEEGESSEVKAVLSDERYQCFKLFTSVFGVGLKTSEKWFRMGFRSLSNIRLDKSLKFTQMQKAGFRYYEDIVSCVTRAEAEAVDVLVNEAVRAFLPDAFITMTGGFRRGKKIGHDVDFLITSPELTEEDEQQLLHKVMNLWEKKGLLLYHDLVESTFEKLKQPSRKVDALDHFQKCFLIFKLYHERVGGDRCRQPEGKDWKAIRVDLVMCPYECHAFALLGWTGSRQFERDLRRYASHERKMILDNHALYDKTKRVFLQAENEEEIFAHLGLDYIEPWERNA

SEQ ID NO: 27 - protein, 379 aa, Ochotona princeps
EYSANPSPGPQATPAVYKISQYACQRRTTLNNHNHIFTDAFEILAENYEFKENEGCYVTYMRAASVLKSLPFTIVSMKDTEGIPCLEDKVKSIMEEIIEEGESSEVKAVLSDERYQCFKLFTSVFGVGLKTSEKWFRMGFRSLSNIRLDKSLKFTQMQKAGFRYYEDIVSCVTRAEAEAVDVLVNEAVRAFLPDAFITMTGGFRRGKKIGHDVDFLITSPELTEEDEQQLLHKVMNLWEKKGLLLYHDLVESTFEKLKQPSRKVDALDHFQKCFLIFKLYHERVGGDRCRQPEGKDWKAIRVDLVMCPYECHAFALLGWTGSRQFERDLRRYASHERKMILDNHALYDKTKRVFLQAENEEEIFAHLGLDYIEPWERNA

SEQ ID NO: 28 - protein, 516 aa, Erinaceus europaeus
MDALPVVHSSPRKKRSRLMGASVAYPPYDIKFHNLVLFILEKKMGSSRRAFLMELARRKGFRVEDELSDSITHIVAENNTGSEVLEWLQVQDIKISSQLELLDVSWLVECMRAGNPVVITGKHQLVSYTVKSDASFGSNPGSQNTPPLAIKKISQYACQRRTSLNNCNHIFTDALDILAENHEFRENEVSCVAFMRAASVLKSLPFTIISMKDTKGIPCLGDKAKCVIEEIIEDGESSEVKAILNDERYQSFKLFTSVFGVGLKTSEKWFRMGFRTLNKIMSDKTLKLTRMQKAGFLYYEDLVSCVAKAEADAVSVLVQEAVWAFLPDAMVTMTGGFRRGKKLGHDVDFLITSPGATEEEEQQLLPKVINFWERKGLLLYHDLVESTFEKLKLPSRKVDALDHFQKCFLILKLHLQHVNGVGNSKTGQQEGKNWKAIRVDLVMCPYERRAFALLGWTGSRQFERDLRRFATHERKMMLDNHALYDKTKRIFLKAESEEEIFAHLGLDYIDPWERNA

SEQ ID NO: 29 - protein, 384 aa, Erinaceus europaeus
DASFGSNPGSQNTPPLAIKKISQYACQRRTSLNNCNHIFTDALDILAENHEFRENEVSCVAFMRAASVLKSLPFTIISMKDTKGIPCLGDKAKCVIEEIIEDGESSEVKAILNDERYQSFKLFTSVFGVGLKTSEKWFRMGFRTLNKIMSDKTLKLTRMQKAGFLYYEDLVSCVAKAEADAVSVLVQEAVWAFLPDAMVTMTGGFRRGKKLGHDVDFLITSPGATEEEEQQLLPKVINFWERKGLLLYHDLVESTFEKLKLPSRKVDALDHFQKCFLILKLHLQHVNGVGNSKTGQQEGKNWKAIRVDLVMCPYERRAFALLGWTGSRQFERDLRRFATHERKMMLDNHALYDKTKRIFLKAESEEEIFAHLGLDYIDPWERNA

SEQ ID NO: 30 - protein, 510 aa, Artificial Sequence
  Tupaia chinensis
  misc_feature (78)..(78): Xaa can be any naturally occurring amino acid
  misc_feature (82)..(82): Xaa can be any naturally occurring amino acid
MDLLRMAPLSPRKKRPRQMGSSMASAPHDIKFQGVVLYILEKKMGTTRRAFLMELARRKGFRVENELSMSLSHQVWDXNCGXDVREWLQVQKVKASSQPELLDVSWLVECMRAGKPVEATGKHQLLVKSDHSTSPSPGPQKTPALAVQKISQYACQRRTTLNNCNRVFTDAFETLAENYEFRENEDSSVIFLRAASVLRSLPFTITSMRDTEGLPCLGDKVKCVIEEIIEDGESSEVNAVLNDERYKSFKLFTSVFGVGLKTSEKWFRMGFRTLSRVRSDKSLHLTRMQQAGFLYYEDLASCVTRAEAEAVGVLVKEAVGAFLPDALVTITGGFRRGKKTGHDVDFLITSPGSTEEKEEELLQKVLNLWEKKGLLLYYDLVESTFEKLKTPSRKVDALDHFPKCFLILKLHHQRVDGDKPSQQEGKSWKAIRVDLVMCPYERHAFALLGWTGSRQFERDLRRYATHERKMMLDNHALYDKTKRVFLKAESEEDIFAHLGLDYIEPWERNA

SEQ ID NO: 31 - protein, 381 aa, Artificial Sequence
  Tupaia chinensis
DHSTSPSPGPQKTPALAVQKISQYACQRRTTLNNCNRVFTDAFETLAENYEFRENEDSSVIFLRAASVLRSLPFTITSMRDTEGLPCLGDKVKCVIEEIIEDGESSEVNAVLNDERYKSFKLFTSVFGVGLKTSEKWFRMGFRTLSRVRSDKSLHLTRMQQAGFLYYEDLASCVTRAEAEAVGVLVKEAVGAFLPDALVTITGGFRRGKKTGHDVDFLITSPGSTEEKEEELLQKVLNLWEKKGLLLYYDLVESTFEKLKTPSRKVDALDHFPKCFLILKLHHQRVDGDKPSQQEGKSWKAIRVDLVMCPYERHAFALLGWTGSRQFERDLRRYATHERKMMLDNHALYDKTKRVFLKAESEEDIFAHLGLDYIEPWERNA

SEQ ID NO: 32 - protein, 525 aa, Ornithorhynchus anatinus
MSFAMFPAKKEHLKKKRRRMNGCISPTLYEIKFNEFVLFILEKKMGTTRRAFLMELARRKGFRVESELSESVTHIVAENNSCSDVLEWLAVQNVGDSSRFELLDISWLTECMKVGKPVEAIGKHQLMRGNCLTNSAPINCMTETPSLATKQVSQYACERRTTLNNCNQKFTDAFEILAKDFEFRENEGICLAFMRAISVLKCLPFTIVRMKDIEGVPWLGDQVKSIIEEIIEDGESSSVKAVLNDERYRSFQLFNSVFEVGLTDNGENGIARGFQTLNEVITDENISLTKTTLSTSLWNYLPGFLYYEDLVSCVAKEEADAVYLIVKEAVRAFLPEALVTLTGGFRRGKKIGHDVDFLISDPESGQDEQLLPNIIKLWEKQELLLYYDLVESTFEKTKIPSRKVDAMDHFQKCFLILKLHHQKVDSGRYKPPPESKNHEAKNWKAIRVDLVMCPFEQYAYALLGWTGSRQFERDLRRYATHEKKMMLDNHALYDKTKKIFLKAESEEDIFTHLGLDYIEPWERNA

SEQ ID NO: 33 - protein, 394 aa, Ornithorhynchus anatinus
LTNSAPINCMTETPSLATKQVSQYACERRTTLNNCNQKFTDAFEILAKDFEFRENEGICLAFMRAISVLKCLPFTIVRMKDIEGVPWLGDQVKSIIEEIIEDGESSSVKAVLNDERYRSFQLFNSVFEVGLTDNGENGIARGFQTLNEVITDENISLTKTTLSTSLWNYLPGFLYYEDLVSCVAKEEADAVYLIVKEAVRAFLPEALVTLTGGFRRGKKIGHDVDFLISDPESGQDEQLLPNIIKLWEKQELLLYYDLVESTFEKTKIPSRKVDAMDHFQKCFLILKLHHQKVDSGRYKPPPESKNHEAKNWKAIRVDLVMCPFEQYAYALLGWTGSRQFERDLRRYATHEKKMMLDNHALYDKTKKIFLKAESEEDIFTHLGLDYIEPWERNA

SEQ ID NO: 34 - protein, 479 aa, Jaculus jaculus
MDPEQAAHWSPRKKRPRQRSASVASAPHDIRFQDLVLFILEKKMGSTRRAFLMELARRKGFRVENELSDSVTHIVAENNSGSDVMKWLQGQNIQASSELELLDVSWLIECMGAGKPVEMTGRHQLVKQTFCLPGFILQDAFDILAENCEFRENEASCVEFMRAASVLKSLPFPIISVKDTEGIPWLGGKVKCVIEEIIEDGESSEVKALLNDERYKSFKLFTSVFGVGLKTAERWFRMGFRTLSTVKLDKSLTFTRMQKAGFLHYEDLVSCVTRAEAEAVSVLVQQAVVAFLPDALVSMTGGFRRGKKIGHDVDFLITSPEATEEEEQQLLHKVTNFWEQKGLLLYCDHVESTFEKCKLPSRKVDALDHFQKCFLILKLYRERVDSVKSSQQEGKGWKAIRVDLVMCPYECRAFALLGWTGSRQFERDLRRYATHERKMRLDNHALYDKTKRVFLKAESEEEIFAHLGLEYIEPLERNA

SEQ ID NO: 35 - protein, 384 aa, Jaculus jaculus
SSELELLDVSWLIECMGAGKPVEMTGRHQLVKQTFCLPGFILQDAFDILAENCEFRENEASCVEFMRAASVLKSLPFPIISVKDTEGIPWLGGKVKCVIEEIIEDGESSEVKALLNDERYKSFKLFTSVFGVGLKTAERWFRMGFRTLSTVKLDKSLTFTRMQKAGFLHYEDLVSCVTRAEAEAVSVLVQQAVVAFLPDALVSMTGGFRRGKKIGHDVDFLITSPEATEEEEQQLLHKVTNFWEQKGLLLYCDHVESTFEKCKLPSRKVDALDHFQKCFLILKLYRERVDSVKSSQQEGKGWKAIRVDLVMCPYECRAFALLGWTGSRQFERDLRRYATHERKMRLDNHALYDKTKRVFLKAESEEEIFAHLGLEYIEPLERNA